European Patent Application EP 4 570 818 A1, published June 18, 2025. Title: HIGHLY TOXIC AMYLOID OLIGOMER AND USE THEREOF. Applicant: Shen Zhen Wisdom Biopharm Co., Ltd. The sequence listing filed with the application follows.

SEQUENCE LISTING (36 sequences)

SEQ ID NO: 1 - DNA, 20 bp, synthetic construct
  source 1..20: mol_type = other DNA
gattatggctcagggtccaa

SEQ ID NO: 2 - DNA, 20 bp, synthetic construct
  source 1..20: mol_type = other DNA
gctccagtgaattcggaaag

SEQ ID NO: 3 - DNA, 20 bp, synthetic construct
  source 1..20: mol_type = other DNA
cccaagcaatacccaaagaa

SEQ ID NO: 4 - DNA, 20 bp, synthetic construct
  source 1..20: mol_type = other DNA
gcttgtgctctgcttgtgag

SEQ ID NO: 5 - DNA, 20 bp, synthetic construct
  source 1..20: mol_type = other DNA
ccggagaggagacttcacag

SEQ ID NO: 6 - DNA, 20 bp, synthetic construct
  source 1..20: mol_type = other DNA
ttgccattgcacaactcttt

SEQ ID NO: 7 - DNA, 20 bp, synthetic construct
  source 1..20: mol_type = other DNA
tgaatacggctacagcaaca

SEQ ID NO: 8 - DNA, 20 bp, synthetic construct
  source 1..20: mol_type = other DNA
aggcccctcctgttattatg

SEQ ID NO: 9 - DNA, 20 bp, synthetic construct
  source 1..20: mol_type = other DNA
cacctggaacagcactctct

SEQ ID NO: 10 - DNA, 20 bp, synthetic construct
  source 1..20: mol_type = other DNA
ctttgtgcgaagtgtcagtg

SEQ ID NO: 11 - DNA, 21 bp, synthetic construct
  source 1..21: mol_type = other DNA
ctggagggtcctttcaacatt

SEQ ID NO: 12 - DNA, 21 bp, synthetic construct
  source 1..21: mol_type = other DNA
gacatcagtaaccagtcggtc

SEQ ID NO: 13 - DNA, 21 bp, synthetic construct
  source 1..21: mol_type = other DNA
tagtcctgtattggcagccac

SEQ ID NO: 14 - DNA, 22 bp, synthetic construct
  source 1..22: mol_type = other DNA
ggctaatgtctatagcagggaa

SEQ ID NO: 15 - DNA, 22 bp, synthetic construct
  source 1..22: mol_type = other DNA
ggtagctggaaatgtggtgcgt

SEQ ID NO: 16 - DNA, 22 bp, synthetic construct
  source 1..22: mol_type = other DNA
gcaccgatgttctccgttgtga

SEQ ID NO: 17 - protein, 5 aa, synthetic construct
SYAMS

SEQ ID NO: 18 - protein, 17 aa, synthetic construct
GISNLGLTTGYADSVKG

SEQ ID NO: 19 - protein, 7 aa, synthetic construct
TTSRFDY

SEQ ID NO: 20 - protein, 11 aa, synthetic construct
RASQSISSYLN

SEQ ID NO: 21 - protein, 7 aa, synthetic construct
KASYLQS

SEQ ID NO: 22 - protein, 9 aa, synthetic construct
QNSAVRPVT

SEQ ID NO: 23 - protein, 242 aa, synthetic construct
MAEVQLLESGGGLVQPGGSLRLSCAASGFTFSSYAMSWVRQAPGKGLEWVSGISNLGLTTGYADSVKGRFTISRDNSKNTLYLQMNSLRAEDTAVYYCAKTTSRFDYWGQGTLVTVSSGGGGSGGGGSGGGGSTDIQMTQSPSSLSASVGDRVTITCRASQSISSYLNWYQQKPGKAPKLLIYKASYLQSGVPSRFSGSGSGTDFTLTISSLQPEDFATYYCQNSAVRPVTFGQGTKVEIKR

SEQ ID NO: 24 - protein, 242 aa, synthetic construct
MAEVQLLESGGGLVQPGGSLRLSCAASGFTFSSYAMSWVRQAPGKGLEWVSGISNLGLTTGYADSVKGRFTISRDNSKNTLYLQMNSLRAEDTAVYYCAKTTSRFDYWGQGTLVTVSSGGGGSGGGGSGGGGSTDIQMTQSPSSLSASVGDRVTITCRASQSISSYLNWYQQKPGKAPKLLIYKASYLQSGVPSRFSGSGSGTDFTLTISSLQPEDFATYYCQQMRRKPVTFGQGTKVEIKR

SEQ ID NO: 25 - protein, 5 aa, synthetic construct
SYAMS

SEQ ID NO: 26 - protein, 17 aa, synthetic construct
GISNLGLTTGYADSVKG

SEQ ID NO: 27 - protein, 7 aa, synthetic construct
TTSRFDY

SEQ ID NO: 28 - protein, 11 aa, synthetic construct
RASQSISSYLN

SEQ ID NO: 29 - protein, 7 aa, synthetic construct
KASYLQS

SEQ ID NO: 30 - protein, 9 aa, synthetic construct
QQMRRKPVT

SEQ ID NO: 31 - protein, 242 aa, synthetic construct
MAEVQLLESGGGLVQPGGSLRLSCAASGFTFSSYAMSWVRQAPGKGLEWVSGISNLGLTTGYADSVKGRFTISRDNSKNTLYLQMNSLRAEDTAVYYCARTTSRFDYWGQGTLVTVSSGGGGSGGGGSGGGGSTDIQMTQSPSSLSASVGDRVTITCRASQSISSYLNWYQQKPGKAPKLLIYKASYLQSGVPSRFSGSGSGTDFTLTISSLQPEDFATYYCQNSAVRPVTFGQGTKVEIKR

SEQ ID NO: 32 - protein, 8 aa, synthetic construct
GFTFSSYA

SEQ ID NO: 33 - protein, 8 aa, synthetic construct
ISNLGLTT

SEQ ID NO: 34 - protein, 9 aa, synthetic construct
AKTTSRFDY

SEQ ID NO: 35 - protein, 6 aa, synthetic construct
QSISSY

SEQ ID NO: 36 - protein, 9 aa, synthetic construct
QNSAVRPVT